European Patent Specification EP 3 356 514 B9, published October 4, 2023. Title: NOUVELLES SOUCHES BACTERIENNES POUR LA PRODUCTION DE VANILLINE. Applicant: Lesaffre et compagnie. The sequence listing filed with the application follows.

SEQUENCE LISTING (10 sequences)

SEQ ID NO: 1 - protein, 540 aa, Amycolatopsis sp.
MGAGRGLPLRQARPVPVRRQGGRPRQGADPVPRPEVLPARPERLRPGEVVRNQGLGSWPVRRARMSPHATAVRHGGTALTYAELSRRVARLANGLRAAGVRPGDRVAYLGPNHPAYLETLFACGQAGAVFVPLNFRLGVPELDHALADSGASVLIHTPEHAETVAALAAGRLLRVPAGELDAADDEPPDLPVGLDDVCLLMYTSGSTGRPKGAMLTHGNLTWNCVNVLVETDLASDERALVAAPLFHAAALGMVCLPTLLKGGTVILHSAFDPGAVLSAVEQERVTLVFGVPTMYQAIAAHPRWRSADLSSLRTLLCGGAPVPADLASRYLDRGLAFVQGYGMTEAAPGVLVLDRAHVAEKIGSAGVPSFFTDVRLAGPSGEPVPPGEKGEIVVSGPNVMKGYWGRPEATAEVLRDGWFHSGDVATVDGDGYFHVVDRLKDMIISGGENIYPAEVENELYGYPGVEACAVIGVPDPRWGEVGKAVVVPADGSRIDGDELLAWLRTRLAGYKVPKSVEFTDRLPTTGSGKILKGEVRRRFG

SEQ ID NO: 2 - protein, 287 aa, Amycolatopsis sp.
MSTAVGNGRVRTEPWGETVLVEFDEGIAWVMLNRPDKRNAMNPTLNDEMVRVLDHLEGDDRCRVLVLTGAGESFSAGMDLKEYFREVDATGSTAVQIKVRRASAEWQWKRLANWSKPTIAMVNGWCFGGAFTPLVACDLAFADEDARFGLSEVNWGIPPGGVVSRALAATVPQRDALYYIMTGEPFDGRRAAEMRLVNEALPADRLRERTREVALKLASMNQVVLHAAKTGYKIAQEMPWEQAEDYLYAKLDQSQFADKAGARAKGLTQFLDQKSYRPGLSAFDPEK

SEQ ID NO: 3 - protein, 613 aa, Phage PhiC31
MTQGVVTGVDTYAGAYDRQSRERENSSAASPATQRSANEDKAADLQREVERDGGRFRFVGHFSEAPGTSAFGTAERPEFERILNECRAGRLNMIIVYDVSRFSRLKVMDAIPIVSELLALGVTIVSTQEGVFRQGNVMDLIHLIMRLDASHKESSLKSAKILDTKNLQRELGGYVGGKAPYGFELVSETKEITRNGRMVNVVINKLAHSTTPLTGPFEFEPDVIRWWWREIKTHKHLPFKPGSQAAIHPGSITGLCKRMDADAVPTRGETIGKKTASSAWDPATVMRILRDPRIAGFAAEVIYKKKPDGTPTTKIEGYRIQRDPITLRPVELDCGPIIEPAEWYELQAWLDGRGRGKGLSRGQAILSAMDKLYCECGAVMTSKRGEESIKDSYRCRRRKVVDPSAPGQHEGTCNVSMAALDKFVAERIFNKIRHAEGDEETLALLWEAARRFGKLTEAPEKSGERANLVAERADALNALEELYEDRAAGAYDGPVGRKHFRKQQAALTLRQQGAEERLAELEAAEAPKLPLDQWFPEDADADPTGPKSWWGRASVDDKRVFVGLFVDKIVVTKSTTGRGQGTPIEKRASITWAKPPTDDDEDDAQDGTEDVAA

SEQ ID NO: 4 - DNA, 39 bp, Phage PhiC31
gccccaactggggtaacctttgagttctctcagttgggg

SEQ ID NO: 5 - DNA, 112 bp, Sphingobium sp.
ccggccagcctcgcagagcaggattcccgttgagcaccgccaggtgcgaataagggacagtgaagaaggaacacccgctcgcgggtgggcctacttcacctatcctgcccgg

SEQ ID NO: 6 - DNA, 1690 bp, Saccharopolyspora erythraea
ggtaccagcccgacccgagcacgcgccggcacgcctggtcgatgtcggaccggagttcgaggtacgcggcttgcaggtccaggaaggggacgtccatgcgagtgtccgttcgagtggcggcttgcgcccgatgctagtcgcggttgatcggcgatcgcaggtgcacgcggtcgatcttgacggctggcgagaggtgcggggaggatctgaccgacgcggtccacacgtggcaccgcgatgctgttgtgggctggacaatcgtgccggttggtaggatccagcggtgagcagttcggacgagcagccgcgcccgcgtcgccgcaaccaggatcggcagcaccccaaccagaaccggccggtgctgggccgtaccgagcgggaccgcaaccggcgccagttcgggcagaacttcctccgcgaccgcaagaccatcgcgcgcatcgccgagacagccgagctgcggcccgatctgccggtgctggaagccggccccgtcgaagggctgctcaccagggaactcgccgaccgcgcgcgtcaggtgacgtcgtacgagatcgacccccggctggcgaagtcgttgcgggagaagctttccggccacccgaacatcgaagtcgtcaacgccgacttcctcaccgccgaaccgccgcccgagccgttcgccttcgtcggcgcgatcccctacggcatcacctcggcgatcgtggactggtgcctggaggcgccgacgatcgagacggcgacgatggtcacgcagctggagttcgcccggaagcggaccggcgattacggccgctggagccgcctcacggtgatgacctggccgctgttcgagtgggagttcgtcgagaaggtcgactcggcgatcatgcggctgcgcaggcgcgccgaaccgctgctggaaggcgcggcgctcgaacgctacgagtcgatggtcgagctgtgcttcaccggcgtcggcggcaacatccaggcgtcgcttctgcgcaagtacccgaggcgccgcgtcgaggcggcgttcgaccacgcgggggtcgggggcggcgccgtggtcgcctacgtccggccggagcagtggctccggctgttcgagcggctggatcagaagaacgaaccgaggggtgggcagccccagcggggcaggcgaaccggcggacgggaccacggggaccggcgaaccggcgggcaggatcgcggcgatcggcgaaccggcggccgcgaccacagggaccggcaagccagcggccacggcgatcgtcgcagcagcggacgcaatcgcgacgacggacgaaccggcgagcgcgagcagggggaccaaggcgggcggcgggggccgtccgggggtggacggaccggcggacgtccagggcgacgcggcggacccgggcagcggtagtccccggcacgcggaacgcggcaggccgtcgagcggcctgccccgttctgtcgagaggaatcagaggttgatgtcggcccggaggtcgatgtcgcgcgacgacgagccgatctccaccgctcgcttgccgcccccgagcttccagccgcccgcggcttcgtcccagtgctggagggccgctccgcgacgtgcacccggacgcgcttggtctcgcccggtgcgagttcgaccttctggtacccggcgagctgtaaatctgccggctcagccttcccaggttcgaatcctggcgcc

SEQ ID NO: 7 - DNA, 27 bp, Artificial Sequence
  Amorce PCR
gaagcttgagcgatgcatgagcacagc

SEQ ID NO: 8 - DNA, 27 bp, Artificial Sequence
  Amorce PCR
gtctagactggttgcgcactacttctc

SEQ ID NO: 9 - DNA, 60 bp, Artificial Sequence
  Amorce PCR
cagctatgacatgattacgaattcgatagcttagcgatgctcacgcagttagacactcac

SEQ ID NO: 10 - DNA, 77 bp, Artificial Sequence
  Amorce PCR
gctccgtccggacccgcccgttgccgaccgctgtgctcatatgtccgctcccttctcccgcgaattcactagtgatt